European Patent Application EP 4 647 771 A1, published November 12, 2025. Title: ANTIBODY OR PEPTIDE BINDING SPECIFICALLY TO RNASE A, AND IMMUNOASSAY APPARATUS AND METHOD FOR SENSING RNASE A, AND METHOD OF COLLECTING RNASE A. Applicant: INDUSTRY-ACADEMIC COOPERATION FOUNDATION, YONSEI UNIVERSITY. Application EP. The sequence listing filed with the application follows.

SEQUENCE LISTING (13 sequences)

SEQ ID NO: 1 - DNA, 75 bp, Synthetic construct
  source 1..75: mol_type = other DNA
gtctattattgcgctcgtnnnnnnnnnnnnnnnnnnnnnnnnnnnnnnnnntggggtcaaggtactacggttacg

SEQ ID NO: 2 - DNA, 22 bp, Synthetic construct
  source 1..22: mol_type = other DNA
cccagttccatgatgccaatgc

SEQ ID NO: 3 - protein, 5 aa, Synthetic construct
TYGIQ

SEQ ID NO: 4 - protein, 17 aa, Synthetic construct
WIHAGTGGTKYSRKFQG

SEQ ID NO: 5 - protein, 11 aa, Synthetic construct
CGPDSDVMTDF

SEQ ID NO: 6 - protein, 11 aa, Synthetic construct
YGPVGRVKRDD

SEQ ID NO: 7 - protein, 11 aa, Synthetic construct
DGTAKKSRKDD

SEQ ID NO: 8 - protein, 120 aa, Synthetic construct
EVQLVESAAEVRRPGASVKITCKASGYSFSTYGIQWMRQAPGQRPEWLGWIHAGTGGTKYSRKFQGRITITRDTSANTVYLDLNSLTSEDTAVYYCARCGPDSDVMTDFWGQGTTVTVSS

SEQ ID NO: 9 - protein, 120 aa, Synthetic construct
EVQLVESAAEVRRPGASVKITCKASGYSFSTYGIQWMRQAPGQRPEWLGWIHAGTGGTKYSRKFQGRITITRDTSANTVYLDLNSLTSEDTAVYYCARYGPVGRVKRDDWGQGTTVTVSS

SEQ ID NO: 10 - protein, 120 aa, Synthetic construct
EVQLVESAAEVRRPGASVKITCKASGYSFSTYGIQWMRQAPGQRPEWLGWIHAGTGGTKYSRKFQGRITITRDTSANTVYLDLNSLTSEDTAVYYCARDGTAKKSRKDDWGQGTTVTVSS

SEQ ID NO: 11 - DNA, 33 bp, Synthetic construct
  source 1..33: mol_type = other DNA
tgtgggccggacagcgacgtgatgacagatttt

SEQ ID NO: 12 - DNA, 33 bp, Synthetic construct
  source 1..33: mol_type = other DNA
tatggtcccgtcggaagagtcaaaagggatgat

SEQ ID NO: 13 - DNA, 33 bp, Synthetic construct
  source 1..33: mol_type = other DNA
gacggaacggctaaaaagagtagaaaggatgat